European Patent Application EP 4 328 313 A1, published February 28, 2024. Title: Adeno-Associated Virus Virion For Treatment of Ornithine Transcarbamylase Deficiency. Applicant: Jichi Medical University Gene Therapy Research Institution Co.,Ltd. The sequence listing filed with the application follows.

SEQUENCE LISTING (18 sequences)

SEQ ID NO: 1 - protein, 735 aa, adeno-associated virus 2 [sequence omitted]

SEQ ID NO: 2 - protein, 736 aa, adeno-associated virus 3A
MAADGYLPDWLEDNLSEGIREWWALKPGVPQPKANQQHQDNRRGLVLPGYKYLGPGNGLDKGEPVNEADAAALEHDKAYDQQLKAGDNPYLKYNHADAEFQERLQEDTSFGGNLGRAVFQAKKRILEPLGLVEEAAKTAPGKKGAVDQSPQEPDSSSGVGKSGKQPARKRLNFGQTGDSESVPDPQPLGEPPAAPTSLGSNTMASGGGAPMADNNEGADGVGNSSGNWHCDSQWLGDRVITTSTRTWALPTYNNHLYKQISSQSGASNDNHYFGYSTPWGYFDFNRFHCHFSPRDWQRLINNNWGFRPKKLSFKLFNIQVRGVTQNDGTTTIANNLTSTVQVFTDSEYQLPYVLGSAHQGCLPPFPADVFMVPQYGYLTLNNGSQAVGRSSFYCLEYFPSQMLRTGNNFQFSYTFEDVPFHSSYAHSQSLDRLMNPLIDQYLYYLNRTQGTTSGTTNQSRLLFSQAGPQSMSLQARNWLPGPCYRQQRLSKTANDNNNSNFPWTAASKYHLNGRDSLVNPGPAMASHKDDEEKFFPMHGNLIFGKEGTTASNAELDNVMITDEEEIRTTNPVATEQYGTVANNLQSSNTAPTTGTVNHQGALPGMVWQDRDVYLQGPIWAKIPHTDGHFHPSPLMGGFGLKHPPPQIMIKNTPVPANPPTTFSPAKFASFITQYSTGQVSVEIEWELQKENSKRWNPEIQYTSNYNKSVNVDFTVDTNGVYSEPRPIGTRYLTRNL

SEQ ID NO: 3 - protein, 736 aa, adeno-associated virus 3B
MAADGYLPDWLEDNLSEGIREWWALKPGVPQPKANQQHQDNRRGLVLPGYKYLGPGNGLDKGEPVNEADAAALEHDKAYDQQLKAGDNPYLKYNHADAEFQERLQEDTSFGGNLGRAVFQAKKRILEPLGLVEEAAKTAPGKKRPVDQSPQEPDSSSGVGKSGKQPARKRLNFGQTGDSESVPDPQPLGEPPAAPTSLGSNTMASGGGAPMADNNEGADGVGNSSGNWHCDSQWLGDRVITTSTRTWALPTYNNHLYKQISSQSGASNDNHYFGYSTPWGYFDFNRFHCHFSPRDWQRLINNNWGFRPKKLSFKLFNIQVKEVTQNDGTTTIANNLTSTVQVFTDSEYQLPYVLGSAHQGCLPPFPADVFMVPQYGYLTLNNGSQAVGRSSFYCLEYFPSQMLRTGNNFQFSYTFEDVPFHSSYAHSQSLDRLMNPLIDQYLYYLNRTQGTTSGTTNQSRLLFSQAGPQSMSLQARNWLPGPCYRQQRLSKTANDNNNSNFPWTAASKYHLNGRDSLVNPGPAMASHKDDEEKFFPMHGNLIFGKEGTTASNAELDNVMITDEEEIRTTNPVATEQYGTVANNLQSSNTAPTTRTVNDQGALPGMVWQDRDVYLQGPIWAKIPHTDGHFHPSPLMGGFGLKHPPPQIMIKNTPVPANPPTTFSPAKFASFITQYSTGQVSVEIEWELQKENSKRWNPEIQYTSNYNKSVNVDFTVDTNGVYSEPRPIGTRYLTRNL

SEQ ID NO: 4 - protein, 736 aa, Artificial Sequence
  AAVGT5 from AAV3B
MAADGYLPDWLEDNLSEGIREWWALKPGVPQPKANQQHQDNRRGLVLPGYKYLGPGNGLDKGEPVNEADAAALEHDKAYDQQLKAGDNPYLKYNHADAEFQERLQEDTSFGGNLGRAVFQAKKRILEPLGLVEEAAKTAPGKKRPVDQSPQEPDSSSGVGKSGKQPARKRLNFGQTGDSESVPDPQPLGEPPAAPTSLGSNTMASGGGAPMADNNEGADGVGNSSGNWHCDSQWLGDRVITTSTRTWALPTYNNHLYKQISSQSGASNDNHYFGYSTPWGYFDFNRFHCHFSPRDWQRLINNNWGFRPKKLSFKLFNIQVKEVTQNDGTTTIANNLTSTVQVFTDSEYQLPYVLGSAHQGCLPPFPADVFMVPQYGYLTLNNGSQAVGRSSFYCLEYFPSQMLRTGNNFQFSYTFEDVPFHSSYAHSQSLDRLMNPLIDQYLYYLNRTQGTTSGTTNQSRLLFSQAGPQSMALQARNWLPGPCYRQQRLSKTANDNNNSNFPWTAASKYHLNGRDSLVNPGPAMASHKDDEEKFFPMHGNLIFGKEGTTASNAELDNVMITDEEEIRTTNPVATEQYGTVANNLQSANTAPTTRTVNDQGALPGMVWQDRDVYLQGPIWAKIPHTDGHFHPSPLMGGFGLKHPPPQIMIKNTPVPANPPTTFSPAKFASFITQYSTGQVSVEIEWELQKENSKRWNPEIQYTSNYAKSVNVDFTVDTNGVYSEPRPIGTRYLTRNL

SEQ ID NO: 5 - protein, 738 aa, adeno-associated virus 8
MAADGYLPDWLEDNLSEGIREWWALKPGAPKPKANQQKQDDGRGLVLPGYKYLGPFNGLDKGEPVNAADAAALEHDKAYDQQLQAGDNPYLRYNHADAEFQERLQEDTSFGGNLGRAVFQAKKRVLEPLGLVEEGAKTAPGKKRPVEPSPQRSPDSSTGIGKKGQQPARKRLNFGQTGDSESVPDPQPLGEPPAAPSGVGPNTMAAGGGAPMADNNEGADGVGSSSGNWHCDSTWLGDRVITTSTRTWALPTYNNHLYKQISNGTSGGATNDNTYFGYSTPWGYFDFNRFHCHFSPRDWQRLINNNWGFRPKRLSFKLFNIQVKEVTQNEGTKTIANNLTSTIQVFTDSEYQLPYVLGSAHQGCLPPFPADVFMIPQYGYLTLNNGSQAVGRSSFYCLEYFPSQMLRTGNNFQFTYTFEDVPFHSSYAHSQSLDRLMNPLIDQYLYYLSRTQTTGGTANTQTLGFSQGGPNTMANQAKNWLPGPCYRQQRVSTTTGQNNNSNFAWTAGTKYHLNGRNSLANPGIAMATHKDDEERFFPSNGILIFGKQNAARDNADYSDVMLTSEEEIKTTNPVATEEYGIVADNLQQQNTAPQIGTVNSQGALPGMVWQNRDVYLQGPIWAKIPHTDGNFHPSPLMGGFGLKHPPPQILIKNTPVPADPPTTFNQSKLNSFITQYSTGQVSVEIEWELQKENSKRWNPEIQYTSNYYKSTSVDFAVNTEGVYSEPRPIGTRYLTRNL

SEQ ID NO: 6 - protein, 624 aa, adeno-associated virus 3A
MPGFYEIVLKVPSDLDERLPGISNSFVNWVAEKEWDVPPDSDMDPNLIEQAPLTVAEKLQREFLVEWRRVSKAPEALFFVQFEKGETYFHLHVLIETIGVKSMVVGRYVSQIKEKLVTRIYRGVEPQLPNWFAVTKTRNGAGGGNKVVDDCYIPNYLLPKTQPELQWAWTNMDQYLSACLNLAERKRLVAQHLTHVSQTQEQNKENQNPNSDAPVIRSKTSARYMELVGWLVDRGITSEKQWIQEDQASYISFNAASNSRSQIKAALDNASKIMSLTKTAPDYLVGSNPPEDITKNRIYQILELNGYDPQYAASVFLGWAQKKFGKRNTIWLFGPATTGKTNIAEAIAHAVPFYGCVNWTNENFPFNDCVDKMVIWWEEGKMTAKVVESAKAILGGSKVRVDQKCKSSAQIEPTPVIVTSNTNMCAVIDGNSTTFEHQQPLQDRMFEFELTRRLDHDFGKVTKQEVKDFFRWASDHVTDVAHEFYVRKGGAKKRPASNDADVSEPKRECTSLAQPTTSDAEAPADYADRYQNKCSRHVGMNLMLFPCKTCERMNQISNVCFTHGQRDCGECFPGMSESQPVSVVKKKTYQKLCPIHHILGRAPEIACSACDLANVDLDDCVSEQ

SEQ ID NO: 7 - protein, 624 aa, adeno-associated virus 3B
MPGFYEIVLKVPSDLDEHLPGISNSFVNWVAEKEWELPPDSDMDPNLIEQAPLTVAEKLQREFLVEWRRVSKAPEALFFVQFEKGETYFHLHVLIETIGVKSMVVGRYVSQIKEKLVTRIYRGVEPQLPNWFAVTKTRNGAGGGNKVVDDCYIPNYLLPKTQPELQWAWTNMDQYLSACLNLAERKRLVAQHLTHVSQTQEQNKENQNPNSDAPVIRSKTSARYMELVGWLVDRGITSEKQWIQEDQASYISFNAASNSRSQIKAALDNASKIMSLTKTAPDYLVGSNPPEDITKNRIYQILELNGYDPQYAASVFLGWAQKKFGKRNTIWLFGPATTGKTNIAEAIAHAVPFYGCVNWTNENFPFNDCVDKMVIWWEEGKMTAKVVESAKAILGGSKVRVDQKCKSSAQIEPTPVIVTSNTNMCAVIDGNSTTFEHQQPLQDRMFKFELTRRLDHDFGKVTKQEVKDFFRWASDHVTDVAHEFYVRKGGAKKRPASNDADVSEPKRQCTSLAQPTTSDAEAPADYADRYQNKCSRHVGMNLMLFPCKTCERMNQISNVCFTHGQRDCGECFPGMSESQPVSVVKKKTYQKLCPIHHILGRAPEIACSACDLANVDLDDCVSEQ

SEQ ID NO: 8 - protein, 624 aa, Artificial Sequence
  baRep protein
MPGFYEIVLKVPSDLDEHLPGISNSFVNWVAEKEWELPPDSDMDPNLIEQAPLTVAEKLQREFLVEWRRVSKAPEALFFVQFEKGETYFHLHVLIETIGVKSMVVGRYVSQIKEKLVTRIYRGVEPQLPNWFAVTKTRNGAGGGNKVVDDCYIPNYLLPKTQPELQWAWTNMDQYLSACLNLAERKRLVAQHLTHVSQTQEQNKENQNPNSDAPVIRSKTSARYMELVGWLVDRGITSEKQWIQEDQASYISFNAASNSRSQIKAALDNASKIMSLTKTAPDYLVGSNPPEDITKNRIYQILELNGYDPQYAASVFLGWAQKKFGKRNTIWLFGPATTGKTNIAEAIAHAVPFYGCVNWTNENFPFNDCVDKMVIWWEEGKMTAKVVESAKAILGGSKVRVDQKCKSSAQIEPTPVIVTSNTNMCAVIDGNSTTFEHQQPLQDRMFEFELTRRLDHDFGKVTKQEVKDFFRWASDHVTDVAHEFYVRKGGAKKRPASNDADVSEPKRECTSLAQPTTSDAEAPADYADRYQNKCSRHVGMNLMLFPCKTCERMNQISNVCFTHGQRDCGECFPGMSESQPVSVVKKKTYQKLCPIHHILGRAPEIACSACDLANVDLDDCVSEQ

SEQ ID NO: 9 - protein, 736 aa, Artificial Sequence
  AAV-LK03 Capsid
MAADGYLPDWLEDNLSEGIREWWALQPGAPKPKANQQHQDNARGLVLPGYKYLGPGNGLDKGEPVNAADAAALEHDKAYDQQLKAGDNPYLKYNHADAEFQERLKEDTSFGGNLGRAVFQAKKRLLEPLGLVEEAAKTAPGKKRPVDQSPQEPDSSSGVGKSGKQPARKRLNFGQTGDSESVPDPQPLGEPPAAPTSLGSNTMASGGGAPMADNNEGADGVGNSSGNWHCDSQWLGDRVITTSTRTWALPTYNNHLYKQISSQSGASNDNHYFGYSTPWGYFDFNRFHCHFSPRDWQRLINNNWGFRPKKLSFKLFNIQVKEVTQNDGTTTIANNLTSTVQVFTDSEYQLPYVLGSAHQGCLPPFPADVFMVPQYGYLTLNNGSQAVGRSSFYCLEYFPSQMLRTGNNFQFSYTFEDVPFHSSYAHSQSLDRLMNPLIDQYLYYLNRTQGTTSGTTNQSRLLFSQAGPQSMSLQARNWLPGPCYRQQRLSKTANDNNNSNFPWTAASKYHLNGRDSLVNPGPAMASHKDDEEKFFPMHGNLIFGKEGTTASNAELDNVMITDEEEIRTTNPVATEQYGTVANNLQSSNTAPTTRTVNDQGALPGMVWQDRDVYLQGPIWAKIPHTDGHFHPSPLMGGFGLKHPPPQIMIKNTPVPANPPTTFSPAKFASFITQYSTGQVSVEIEWELQKENSKRWNPEIQYTSNYNKSVNVDFTVDTNGVYSEPRPIGTRYLTRPL

SEQ ID NO: 10 - DNA, 1065 bp, Homo sapiens
  CDS (1)..(1065)
atgctgttcaacctgcggatcctgctgaacaacgccgccttcagaaacggccacaacttcatggtccgaaacttcagatgcggccagcctctgcagaacaaggtgcagctgaagggcagagatctgctgaccctgaagaacttcaccggcgaagagatcaagtacatgctgtggctgagcgccgacctgaagttccggattaagcagaagggcgagtacctgcctctgctgcagggaaagtctctgggcatgatcttcgagaagcggagcaccagaaccagactgagcaccgagacaggctttgccctgctcggaggacacccctgctttctgacaacccaggacatccacctgggcgtgaacgagagcctgaccgatacagccagagtgctgagcagcatggctgatgccgtgctggccagagtgtacaagcagagcgatctggacaccctggccaaagaggccagcattcccatcatcaacggcctgagcgacctgtatcaccccatccagatcctggccgactacctgacactgcaagagcactacagcagcctgaagggactgaccctgtcttggatcggcgacggcaacaacatcctgcactctatcatgatgagcgccgccaagttcggcatgcatctgcaggccgctacacccaagggctatgagcctgatgccagcgtgacaaagctggccgagcagtacgccaaagagaacggcacaaagctgctgctgaccaacgatcccctggaagctgcccatggcggcaatgtgctgatcaccgatacctggatcagcatgggccaagaggaagagaagaagaagcggctgcaggccttccagggctaccaagtgacaatgaagaccgccaaggtggccgccagcgattggacctttctgcactgcctgcctcggaagcctgaagaggtggacgacgaggtgttctacagccctagaagcctggtgttccccgaggccgagaacagaaagtggaccatcatggctgtgatggtgtccctgctgaccgactactctccccagctgcagaaacccaagttctga

SEQ ID NO: 11 - protein, 354 aa, Homo sapiens
MLFNLRILLNNAAFRNGHNFMVRNFRCGQPLQNKVQLKGRDLLTLKNFTGEEIKYMLWLSADLKFRIKQKGEYLPLLQGKSLGMIFEKRSTRTRLSTETGFALLGGHPCFLTTQDIHLGVNESLTDTARVLSSMADAVLARVYKQSDLDTLAKEASIPIINGLSDLYHPIQILADYLTLQEHYSSLKGLTLSWIGDGNNILHSIMMSAAKFGMHLQAATPKGYEPDASVTKLAEQYAKENGTKLLLTNDPLEAAHGGNVLITDTWISMGQEEEKKKRLQAFQGYQVTMKTAKVAASDWTFLHCLPRKPEEVDDEVFYSPRSLVFPEAENRKWTIMAVMVSLLTDYSPQLQKPKF

SEQ ID NO: 12 - DNA, 3534 bp, Artificial Sequence
  AAV.GT5-HCRhAAT promoter- human OTC-WPRE
  misc_feature (1)..(146): Inverted Terminal Repeat
  misc_feature (397)..(1046): HCRhAAT promoter
  misc_feature (1173)..(2237): OTC cDNA
  misc_feature (2497)..(3085): WPRE
  misc_feature (3179)..(3300): SV40 polyA
  misc_feature (3390)..(3534): Inverted Terminal Repeat
ttggccactccctctatgcgcactcgctcgctcggtggggccggacgtgcaaagcacgtccgtctggcgacctttggtcgccaggccccaccgagcgagcgagtgcgcatagagggagtggccaactccatcactagaggtatggcagtgacgtaacgcgaagcgcgcgaagcgagaccatgaattatcctgctgatgaagcagaacaactttaacgccgtgcgctgttcgcattatccgaaccatccgctgtggtacacgctgtgcgaccgctacggcctgtatgtggtggatgaagccaatattgaaacccacggcatggtgccaatgaatcgtctgaccgatgatccgcgctggctaccggcgatgagcgaacgcggccgcacgcgtactagtctgcaggctcagaggcacacaggagtttctgggctcaccctgcccccttccaacccctcagttcccatcctccagcagctgtttgtgtgctgcctctgaagtccacactgaacaaacttcagcctactcatgtccctaaaatgggcaaacattgcaagcagcaaacagcaaacacacagccctccctgcctgctgaccttggagctggggcagaggtcagagacctctctgggcccatgccacctccaacatccactcgaccccttggaatttcggtggagaggagcagaggttgtcctggcgtggtttaggtagtgtgagagggtccgggttcaagggcgaattcgccctcagagactgtctgactcacgccaccccctccaccttggacacaggacgctgtggtttctgagccaggtacaatgactcctttcggtaagtgcagtggaagctgtacactgcccaggcaaagcgtccgggcagcgtaggcgggcgactcagatcccagccagtggacttagcccctgtttgctcctccgataactggggtgaccttggttaatattcaccagcagcctcccccgttgcccctctggatccactgcttaaatacggacgaggacagggccctgtctcctcagcttcaggcagggcgaattccccggggatcctctagaaacacatttcttagtttttaggtggcccccgctggctaacttgctgtggagttttcaagggcatagaatcgtcctttacacaattaaaagaaggccaccatgctgttcaacctgcggatcctgctgaacaacgccgccttcagaaacggccacaacttcatggtccgaaacttcagatgcggccagcctctgcagaacaaggtgcagctgaagggcagagatctgctgaccctgaagaacttcaccggcgaagagatcaagtacatgctgtggctgagcgccgacctgaagttccggattaagcagaagggcgagtacctgcctctgctgcagggaaagtctctgggcatgatcttcgagaagcggagcaccagaaccagactgagcaccgagacaggctttgccctgctcggaggacacccctgctttctgacaacccaggacatccacctgggcgtgaacgagagcctgaccgatacagccagagtgctgagcagcatggctgatgccgtgctggccagagtgtacaagcagagcgatctggacaccctggccaaagaggccagcattcccatcatcaacggcctgagcgacctgtatcaccccatccagatcctggccgactacctgacactgcaagagcactacagcagcctgaagggactgaccctgtcttggatcggcgacggcaacaacatcctgcactctatcatgatgagcgccgccaagttcggcatgcatctgcaggccgctacacccaagggctatgagcctgatgccagcgtgacaaagctggccgagcagtacgccaaagagaacggcacaaagctgctgctgaccaacgatcccctggaagctgcccatggcggcaatgtgctgatcaccgatacctggatcagcatgggccaagaggaagagaagaagaagcggctgcaggccttccagggctaccaagtgacaatgaagaccgccaaggtggccgccagcgattggacctttctgcactgcctgcctcggaagcctgaagaggtggacgacgaggtgttctacagccctagaagcctggtgttccccgaggccgagaacagaaagtggaccatcatggctgtgatggtgtccctgctgaccgactactctccccagctgcagaaacccaagttctgatgttgtgttacttgtcaagaaagaagcaatgttcttcagtaacagaatgagttggtttatggggaaaagagaagagaatctaaaaaataaacaaatccctaacacgtggtatgggtgaaccgtatgatatgctttgccattgtgaaactttccttaagcctttaatttaagtgctgatgcactgtaatacgtgcttaactttgcttaaactctctaattcccaatttctgagttacatttagatatcaagcttatcgataatcaacctctggattacaaaatttgtgaaagattgactggtattcttaactatgttgctccttttacgctatgtggatacgctgctttaatgcctttgtatcatgctattgcttcccgtatggctttcattttctcctccttgtataaatcctggttgctgtctctttatgaggagttgtggcccgttgtcaggcaacgtggcgtggtgtgcactgtgtttgctgacgcaacccccactggttggggcattgccaccacctgtcagctcctttccgggactttcgctttccccctccctattgccacggcggaactcatcgccgcctgccttgcccgctgctggacaggggctcggctgttgggcactgacaattccgtggtgttgtcggggaaatcatcgtcctttccttggctgctcgcctgtgttgccacctggattctgcgcgggacgtccttctgctacgtcccttcggccctcaatccagcggaccttccttcccgcggcctgctgccggctctgcggcctcttccgcgtcttcgccttcgccctcagacgagtcggatctccctttgggccgcctccccgcatcgataccgtcgacctcgaggcaagcttgggcccggtacccaattcgccctatagtgagtcgtattacgcgcgcagcggccgaccatggcccaacttgtttattgcagcttataatggttacaaataaagcaatagcatcacaaatttcacaaataaagcatttttttcactgcattctagttgtggtttgtccaaactcatcaatgtatcttatcatgtctggatctccggacactagataagcagcggcctgcggcgcttgcgcttcgcggtttacaactgctggttaatatttaactctcgccatacctctagtgatggagttggccactccctctatgcgcactcgctcgctcggtggggcctggcgaccaaaggtcgccagacggacgtgctttgcacgtccggccccaccgagcgagcgagtgcgcatagagggagtggcca

SEQ ID NO: 13 - DNA, 20 bp, Artificial Sequence
  OTC Forward
accggcgaagagatcaagta

SEQ ID NO: 14 - DNA, 20 bp, Artificial Sequence
  OTC Reverse
atcatgcccagagactttcc

SEQ ID NO: 15 - DNA, 20 bp, Artificial Sequence
  GAPDH Forward
aattccatggcaccgtcaag

SEQ ID NO: 16 - DNA, 20 bp, Artificial Sequence
  GAPDH Reverse
atcgccccacttgattttgg

SEQ ID NO: 17 - protein, 736 aa, Artificial Sequence
  AAV.M1 (S587A)
MAADGYLPDWLEDNLSEGIREWWALKPGVPQPKANQQHQDNRRGLVLPGYKYLGPGNGLDKGEPVNEADAAALEHDKAYDQQLKAGDNPYLKYNHADAEFQERLQEDTSFGGNLGRAVFQAKKRILEPLGLVEEAAKTAPGKKRPVDQSPQEPDSSSGVGKSGKQPARKRLNFGQTGDSESVPDPQPLGEPPAAPTSLGSNTMASGGGAPMADNNEGADGVGNSSGNWHCDSQWLGDRVITTSTRTWALPTYNNHLYKQISSQSGASNDNHYFGYSTPWGYFDFNRFHCHFSPRDWQRLINNNWGFRPKKLSFKLFNIQVKEVTQNDGTTTIANNLTSTVQVFTDSEYQLPYVLGSAHQGCLPPFPADVFMVPQYGYLTLNNGSQAVGRSSFYCLEYFPSQMLRTGNNFQFSYTFEDVPFHSSYAHSQSLDRLMNPLIDQYLYYLNRTQGTTSGTTNQSRLLFSQAGPQSMSLQARNWLPGPCYRQQRLSKTANDNNNSNFPWTAASKYHLNGRDSLVNPGPAMASHKDDEEKFFPMHGNLIFGKEGTTASNAELDNVMITDEEEIRTTNPVATEQYGTVANNLQSANTAPTTRTVNDQGALPGMVWQDRDVYLQGPIWAKIPHTDGHFHPSPLMGGFGLKHPPPQIMIKNTPVPANPPTTFSPAKFASFITQYSTGQVSVEIEWELQKENSKRWNPEIQYTSNYNKSVNVDFTVDTNGVYSEPRPIGTRYLTRNL

SEQ ID NO: 18 - protein, 736 aa, Artificial Sequence
  AAV.M2 (S472A, S587A)
MAADGYLPDWLEDNLSEGIREWWALKPGVPQPKANQQHQDNRRGLVLPGYKYLGPGNGLDKGEPVNEADAAALEHDKAYDQQLKAGDNPYLKYNHADAEFQERLQEDTSFGGNLGRAVFQAKKRILEPLGLVEEAAKTAPGKKRPVDQSPQEPDSSSGVGKSGKQPARKRLNFGQTGDSESVPDPQPLGEPPAAPTSLGSNTMASGGGAPMADNNEGADGVGNSSGNWHCDSQWLGDRVITTSTRTWALPTYNNHLYKQISSQSGASNDNHYFGYSTPWGYFDFNRFHCHFSPRDWQRLINNNWGFRPKKLSFKLFNIQVKEVTQNDGTTTIANNLTSTVQVFTDSEYQLPYVLGSAHQGCLPPFPADVFMVPQYGYLTLNNGSQAVGRSSFYCLEYFPSQMLRTGNNFQFSYTFEDVPFHSSYAHSQSLDRLMNPLIDQYLYYLNRTQGTTSGTTNQSRLLFSQAGPQSMALQARNWLPGPCYRQQRLSKTANDNNNSNFPWTAASKYHLNGRDSLVNPGPAMASHKDDEEKFFPMHGNLIFGKEGTTASNAELDNVMITDEEEIRTTNPVATEQYGTVANNLQSANTAPTTRTVNDQGALPGMVWQDRDVYLQGPIWAKIPHTDGHFHPSPLMGGFGLKHPPPQIMIKNTPVPANPPTTFSPAKFASFITQYSTGQVSVEIEWELQKENSKRWNPEIQYTSNYNKSVNVDFTVDTNGVYSEPRPIGTRYLTRNL